European Patent Application EP 4 491 636 A1, published January 15, 2025. Title: Antibody targeting cotinine or antigen-binding fragment thereof, and Chimeric antigen receptor comprising the same, and Uses thereof. Applicant: AbClon Inc. The sequence listing filed with the application follows.

SEQUENCE LISTING (17 sequences)

SEQ ID NO: 1 - protein, 5 aa, synthetic construct
SYWIQ

SEQ ID NO: 2 - protein, 17 aa, synthetic construct
EIFPGTGTTYYNEKFKG

SEQ ID NO: 3 - protein, 13 aa, synthetic construct
GGYYYDSRAWFAY

SEQ ID NO: 4 - protein, 14 aa, synthetic construct
RSSTGTVTTSNYAN

SEQ ID NO: 5 - protein, 7 aa, synthetic construct
GTNNRAP

SEQ ID NO: 6 - protein, 9 aa, synthetic construct
ALWFSNHWV

SEQ ID NO: 7 - protein, 122 aa, synthetic construct
EVQLQQSGAELVKPGASVKLSCKTSGYTFTSYWIQWIKQRPGQGLGWVGEIFPGTGTTYYNEKFKGKATLTIDTSSSTAYMQLSSLTSEDSAVYFCARGGYYYDSRAWFAYWGQGTLVTVSA

SEQ ID NO: 8 - protein, 110 aa, synthetic construct
DAVVTQESALTTSPGETVTLTCRSSTGTVTTSNYANWVQEKPDHLFTGLIGGTNNRAPGVPARFSGSLIGDEAALTITGAQTEDEAIYFCALWFSNHWVFGGGTKLTVLG

SEQ ID NO: 9 - protein, 122 aa, synthetic construct
QVQLVQSGAEVKKPGASVKVSCKASGYTFTSYWIQWVRQAPGQGLEWMGEIFPGTGTTYYNEKFKGRVTMTIDTSTSTVYMELSSLRSEDTAVYYCARGGYYYDSRAWFAYWGQGTLVTVSS

SEQ ID NO: 10 - protein, 110 aa, synthetic construct
QAVVTQEPSLTVSPGGTVTLTCRSSTGTVTTSNYANWVQQKPGQAPRGLIGGTNNRAPWTPARFSGSLLGDKAALTLSGAQPEDEAEYYCALWFSNHWVFGGGTKLTVLG

SEQ ID NO: 11 - protein, 20 aa, synthetic construct
METDTLLLWVLLLWVPGSTG

SEQ ID NO: 12 - DNA, 367 bp, synthetic construct
  source 1..367: mol_type = other DNA
gaggtgcagcttcagcagtctggagctgagctggtgaagcctggggcttcagtgaagctgtcctgcaagacttctggctacaccttcaccagctactggattcagtggataaaacagaggcctggacagggccttgggtgggttggagagatatttcctggaactggcactacttactacaatgagaagttcaagggcaaggccacactgactatagacacatcctccagcacagcctacatgcagctcagcagcctgacctctgaggactctgctgtctatttctgtgcaagagggggttattactacgatagtagagcctggtttgcttactggggccaagggactctggtcactgtctctgcag

SEQ ID NO: 13 - DNA, 330 bp, synthetic construct
  source 1..330: mol_type = other DNA
gatgctgttgtgactcaggaatctgcactcaccacatcacctggtgaaacagtcacactcacttgtcgctcaagtactgggactgttacaactagtaactatgccaactgggtccaagaaaaaccagatcatttattcactggtctaataggtggtaccaacaaccgagctccaggtgttcctgccagattctcaggctccctgattggagacgaggctgccctcaccatcacaggggcacagactgaagatgaggcaatatatttctgtgctctatggttcagcaaccattgggtgttcggtggaggaaccaaactgactgtcctaggt

SEQ ID NO: 14 - DNA, 366 bp, synthetic construct
  source 1..366: mol_type = other DNA
caagtgcagttggtccagtcaggcgcagaagtaaagaaaccaggagcgtcagttaaggtcagctgcaaggcgagcggctatacgttcacttcatattggattcagtgggtacggcaagcgcctggtcagggcttggaatggatgggcgaaatttttcctgggaccgggacgacatattacaacgaaaagttcaagggaagagttaccatgacgatcgatacatctaccagtacagtctacatggaacttagcagtcttaggagcgaggatacagcagtatattattgtgcgagaggtggatactactatgatagccgggcgtggttcgcgtattggggccaggggacacttgtgaccgtcagtagt

SEQ ID NO: 15 - DNA, 330 bp, synthetic construct
  source 1..330: mol_type = other DNA
caagcggttgtgacacaagagccctctttgactgtaagcccgggtggtacggtcacacttacatgccgcagctctaccgggactgtaacaaccagcaactacgcgaactgggtacaacagaaacctggacaagcgccacgcggtttgataggagggacgaataatcgcgccccttggacccctgcgagattctctggatctttgcttggggacaaagcagcccttacccttagcggcgcacagccagaggatgaagctgagtattattgcgcgctgtggttttcaaaccactgggtgttcggcggcggcacgaaattgaccgttcttggg

SEQ ID NO: 16 - DNA, 1184 bp, synthetic construct
  source 1..1184: mol_type = other DNA
tgtgaggctccggtgcccgtcagtgggcagagcgcacatcgcccacagtccccgagaagttggggggaggggtcggcaattgaaccggtgcctagagaaggtggcgcggggtaaactgggaaagtgatgtcgtgtactggctccgcctttttcccgagggtgggggagaaccgtatataagtgcagtagtcgccgtgaacgttctttttcgcaacgggtttgccgccagaacacaggtaagtgccgtgtgtggttcccgcgggcctggcctctttacgggttatggcccttgcgtgccttgaattacttccacctggctgcagtacgtgattcttgatcccgagcttcgggttggaagtgggtgggagagttcgaggccttgcgcttaaggagccccttcgcctcgtgcttgagttgaggcctggcctgggcgctggggccgccgcgtgcgaatctggtggcaccttcgcgcctgtctcgctgctttcgataagtctctagccatttaaaatttttgatgacctgctgcgacgctttttttctggcaagatagtcttgtaaatgcgggccaagatctgcacactggtatttcggtttttggggccgcgggcggcgacggggcccgtgcgtcccagcgcacatgttcggcgaggcggggcctgcgagcgcggccaccgagaatcggacgggggtagtctcaagctggccggcctgctctggtgcctggcctcgcgccgccgtgtatcgccccgccctgggcggcaaggctggcccggtcggcaccagttgcgtgagcggaaagatggccgcttcccggccctgctgcagggagctcaaaatggaggacgcggcgctcgggagagcgggcgggtgagtcacccacacaaaggaaaagggcctttccgtcctcagccgtcgcttcatgtgactccacggagtaccgggcgccgtccaggcacctcgattagttctcgagcttttggagtacgtcgtctttaggttggggggaggggttttatgcgatggagtttccccacactgagtgggtggagactgaagttaggccagcttggcacttgatgtaattctccttggaatttgccctttttgagtttggatcttggttcattctcaagcctcagacagtggttcaaagtttttttcttccatttcaggtgtcgtga

SEQ ID NO: 17 - DNA, 651 bp, synthetic construct
  source 1..651: mol_type = other DNA
atcgaggtgatgtaccctcctccctatctcgataacgagaaatctaacggcaccatcatccatgtgaaagggaaacacctctgcccttcaccactcttcccaggtccgagcaagccaatttatatctgggcaccgttggcggggacttgcggagtgcttttactttcactggttattacgctgtactgtaaacgcggtcggaagaagctcctttacattttcaagcagccttttatgcgcccagtgcagaccacacaggaggaagatggctgtagttgcagatttcccgaggaagaagagggagggtgtgaactgagagtcaaattcagccgttccgctgatgccccagcctatcaacaggggcagaatcaactgtataatgaattgaatctgggcaggagagaagaatacgacgtcctggataagaggcgaggcagagaccccgagatgggcggtaaaccccggcggaagaacccccaggaaggcctgtacaacgagctgcagaaggacaagatggctgaggcctactccgaaataggaatgaagggggagagaaggagaggcaaaggacatgacggcctgtaccagggactgtctacagctactaaggacacctatgatgcattgcacatgcaagccctaccccctaga